European Patent Application EP 4 239 067 A2, published September 6, 2023. Title: TRANSPOSASE COMPOSITIONS FOR REDUCTION OF INSERTION BIAS. Applicant: Illumina Inc. Application EP. The sequence listing filed with the application follows.

SEQUENCE LISTING (7 sequences)

SEQ ID NO: 1 - DNA, 51 bp, synthetic construct
  misc_feature 1..51: note = Figure 15 HyperMu
  source 1..51: mol_type = other DNA
tgttttcgcatttatcgtgaaacgctttcgcgtttttcgtgccccgcttca

SEQ ID NO: 2 - DNA, 56 bp, synthetic construct
  misc_feature 1..56: note = Figure 15 HyperMu
  source 1..56: mol_type = other DNA
tcggatgaagcggggcacgaaaaacgcgaaagcgtttcacgataaatgcgaaaaca

SEQ ID NO: 3 - DNA, 51 bp, synthetic construct
  misc_feature 1..51: note = Figure 16 MM1141
  source 1..51: mol_type = other DNA
tgttttcgcatttatcgtgaaacgctttcgcgtttttcgtgcgccgcttca

SEQ ID NO: 4 - DNA, 56 bp, synthetic construct
  misc_feature 1..56: note = Figure 16 MM1138
  source 1..56: mol_type = other DNA
tcggatgaagcggcgcacgaaaaacgcgaaagcgtttcacgataaatgcgaaaaca

SEQ ID NO: 5 - DNA, 21 bp, synthetic construct
  misc_feature 1..21: note = Figure 16 Sequencing primer
  source 1..21: mol_type = other DNA
cgtttttcgtgcgccgcttca

SEQ ID NO: 6 - DNA, 45 bp, synthetic construct
  misc_feature 1..45: note = Figure 16 P7MUTS
  source 1..45: mol_type = other DNA
caagcagaagacggcatacgagatcgtttttcgtgcgccgcttca

SEQ ID NO: 7 - DNA, 50 bp, synthetic construct
  misc_feature 1..50: note = Figure 16 P5MUTS
  source 1..50: mol_type = other DNA
aatgatacggcgaccaccgagatctacaccgtttttcgtgcgccgcttca